European Patent Application EP 4 624 497 A1, published October 1, 2025. Title: Phosphoenolpyruvate optical probe, preparation method therefor and application thereof. Applicant: EAST CHINA UNIVERSITY OF SCIENCE AND TECHNOLOGY. Application EP EP23893907.8, filed November 22, 2023. The sequence listing filed with the application follows.

SEQUENCE LISTING (13 sequences)

SEQ ID NO: 1 - protein, 322 aa, synthetic construct
MKRIGVFTSGGDAPGMNAAIRAVVRQAHALGVEVIGIRRGYAGMIQGEMVPLGVRDVANIIQRGGTILLTARSQEFLTEEGRAKAYAKLQAAGIEGLVAIGGDGTFRGALFLVEEHGMPVVGVPGTIDNDLYGTDYTIGFDTAVNTALEAIDRIRDTAASHERVFFIEVMGRHAGFIALDVGLAGGAEVIAVPEEPVDPKAVAEVLEASQRRGKKSSIVVVAEGAYPGGAAGLLAAIREHLQVEARVTVLGHIQRGGSPTAKDRILASRLGAPAVEALVGGASGVMVGEVEGEVDLTPLKEAVERRKDINRALLRLSQVLAL

SEQ ID NO: 2 - protein, 246 aa, synthetic construct
YNSDNVYIMADKQKNGIKANFKIRHNVEDGSVQLADHYQQNTPIGDGPVLLPDNHYLSFQSVLSKDPNEKRDHMVLLEFVTAAGITLGMDELYNVDGGSGGTGSKGEELFTGVVPILVELDGDVNGHKFSVSGEGEGDATYGKLTLKLICTTGKLPVPWPTLVTTLGYGLKCFARYPDHMKQHDFFKSAMPEGYVQERTIFFKDDGNYKTRAEVKFEGDTLVNRIELKGIDFKEDGNILGHKLEYN

SEQ ID NO: 3 - protein, 242 aa, synthetic construct
VSERMYPEDGVLKSEIKKGLRLKDGGHYAAEVKTTYKAKKPVQLPGAYIVDIKLDIVSHNEDYTIVEQCERAEGRHPTGGRDELYKGGTGGSLVSKGEEDNMAIIKEFMRFKVHMEGSVNGHEFEIEGEGEGRPYEAFQTAKLKVTKGGPLPFAWDILSPQFTYGSKAYIKHPADIPDYFKLSFPEGFRWERVMNFEDGGIIHVNQDSSLQDGVFIYKVKLRGTNFPPDGPVMQKKTMGWEA

SEQ ID NO: 4 - protein, 250 aa, synthetic construct
MGGRSKKPAKNLKMPGVYYVDRRLERIKEADKETYVEQHEVAVARYCDLPSKLGHKLNGGTGGSMVSKGEELIKENMHMKLYMEGTVNNHHFKCTSEGEGKPYEGTQTMRIKVVEGGPLPFAFDILATSFMYGSKTFINHTQGIPDFFKQSFPEGFTWERVTTYEDGGVLTATQDTSLQDGCLIYNVKIRGVNFPSNGPVMQKKTLGWEASTEMLYPADGGLEGRSDMALKLVGGGHLICNLKTTYRSKK

SEQ ID NO: 5 - protein, 236 aa, synthetic construct
MVSKGEEDNMAIIKEFMRFKVHMEGSVNGHEFEIEGEGEGRPYEGTQTAKLKVTKGGPLPFAWDILSPQFMYGSKAYVKHPADIPDYLKLSFPEGFKWERVMNFEDGGVVTVTQDSSLQDGEFIYKVKLRGTNFPSDGPVMQKKTMGWEASSERMYPEDGALKGEIKQRLKLKDGGHYDAEVKTTYKAKKPVQLPGAYNVNIKLDITSHNEDYTIVEQYERAEGRHSTGGMDELYK

SEQ ID NO: 6 - protein, 241 aa, synthetic construct
NVYIKADKQKNGIKANFKIRHNIEDGGVQLAYHYQQNTPIGDGPVLLPDNHYLSVQSILSKDPNEKRDHMVLLEFVTAAGITLGMDELYKGGTGGSMVSKGEELFTGVVPIQVELDGDVNGHKFSVSGEGEGDATYGKLTLKFICTTGKLPVPWPTLVTTLTYGVQCFSRYPDHMKQHDFFKSAMPEGYIQERTIFFKDDGNYKTRAEVKFEGDTLVNRIELKGIDFKEDGNILGHKLEYN

SEQ ID NO: 7 - protein, 243 aa, synthetic construct
NVYIKADKQKNGIKANFKIRHNIEGGGVQLAYHYQQNTPIGDGPVLLPDNHYLSVQSILSKDPNEKRDHMVLLEFVTAAGITLGMDELYKGGTGGSESMVSKGEELFTGVVPIQVELDGDVNGHKFSVSGEGEGDATYGKLTLKFICTTGKLPVPWPTLVTTLSHGVQCFSRYPDHMKQHDFFKSAMPGGYIQERTIFFKDDGNYKTRAEVKFEGDTLVNRIELKGIDFKEDGNILGHKLEYN

SEQ ID NO: 8 - protein, 233 aa, synthetic construct
MSELITENMHMKLYMEGTVNNHHFKCTSEGEGKPYEGTQTMRIKVVEGGPLPFAFDILATSFMYGSKTFINHTQGIPDFFKQSFPEGFTWERVTTYEDGGVLTATQDTSLQDGCLIYNVKIRGVNFPSNGPVMQKKTLGWEASTEMLYPADGGLEGRADMALKLVGGGHLICNLKTTYRSKKPAKNLKMPGVYYVDRRLERIKEADKETYVEQHEVAVARYCDLPSKLGHKLN

SEQ ID NO: 9 - protein, 242 aa, synthetic construct
VSERMYPEDGALKSEIKKGLRLKDGGHYAAEVKTTYKAKKPVQLPGAYIVDIKLDIVSHNEDYTIVEQCERAEGRHSTGGMDELYKGGTGGSLVSKGEEDNMAIIKEFMRFKVHMEGSVNGHEFEIEGEGEGRPYEAFQTAKLKVTKGGPLPFAWDILSPQFMYGSKAYIKHPADIPDYFKLSFPEGFRWERVMNFEDGGIIHVNQDSSLQDGVFIYKVKLRGTNFPPDGPVMQKKTMGWEA

SEQ ID NO: 10 - protein, 568 aa, synthetic construct
MKRIGVFTSGGDAPGMNAAIRAVVRQAHALGVEVIGIRRGYAGMIQGEMVPLGVRDVANIIQRGGTILLTARSQEFLTEEGRAKAYAKLQAAGIEGLVAIGGDGTFRGALFLVEEHGMPVVGVPGTIDNDLYGTDYTIGFDTAVNTALEAIDRIRDTAASHERVFFIEVMGRHAGFIALDVGLAGGAEVIAVPEEPVDPKAVAEVLEASQRRGKKSSIVVVAEGAYPGGAAGLLAAIREHLQVEARVTVLGHIQYNSDNVYIMADKQKNGIKANFKIRHNVEDGSVQLADHYQQNTPIGDGPVLLPDNHYLSFQSVLSKDPNEKRDHMVLLEFVTAAGITLGMDELYNVDGGSGGTGSKGEELFTGVVPILVELDGDVNGHKFSVSGEGEGDATYGKLTLKLICTTGKLPVPWPTLVTTLGYGLKCFARYPDHMKQHDFFKSAMPEGYVQERTIFFKDDGNYKTRAEVKFEGDTLVNRIELKGIGFKEDGNILGHKLEYNRGGSPTAKDRILASRLGAPAVEALVGGASGVMVGEVEGEVDLTPLKEAVERRKDINRALLRLSQVLAL

SEQ ID NO: 11 - DNA, 1704 bp, synthetic construct
  source 1..1704: mol_type = other DNA
atgaaacgcattggcgtgtttaccagcggtggtgatgcgcctggtatgaatgcggcgattcgtgcggttgttcgtcaggcgcatgcgttaggcgttgaagtgattggcattcgccgtggctatgcgggtatgattcagggtgaaatggtgcctttaggcgtgcgtgatgtggcgaacattattcaacgcggcggcaccattttattaaccgcgcgcagccaagaatttctgaccgaagaaggccgcgcaaaagcgtatgcgaaactgcaggcggcgggtattgaaggtctggtggcgattggtggtgatggaacctttcgtggcgcgctgtttctggtggaagaacatggcatgccggttgtgggtgtgcctggaaccattgataacgatctgtacggcaccgattataccattggctttgataccgcggttaacacagccctggaagcgattgatcgcattcgtgataccgcggcgtcacatgaacgcgtgtttttcattgaagtgatgggccgccatgcgggttttattgcgctggatgttggcttagcaggcggtgcggaagttattgcggtgccggaagaacctgtggacccgaaagcggtggcggaagttttagaagcgagccaacgccgtggcaaaaaaagcagcattgtggtggttgcggaaggtgcatatcctggtggcgcggcgggtttattagcggcgattcgcgaacatctgcaggttgaagcgcgcgttaccgtgttaggccatattcagtacaacagcgacaacgtctatatcatggccgacaagcagaagaacggcatcaaggccaacttcaagatccgccacaacgtcgaggacggcagcgtgcagctcgccgaccactaccagcagaacacccccatcggcgacggccccgtgctgctgcccgacaaccactacctgagcttccagtccgtcctgagcaaagaccccaacgagaagcgcgatcacatggtcctgctggagttcgtgaccgccgccgggatcactctcggcatggacgagctgtacaacgtggatggcggtagcggtggcaccggcagcaagggcgaggagctgttcaccggggtggtgcccatcctggtcgagctggacggcgacgtaaacggccacaagttcagcgtgtccggcgagggcgagggcgatgccacctacggcaagctgaccctgaagctgatctgcaccaccggcaagctgcccgtgccctggcccaccctcgtgaccaccctcggctacggcctgaagtgcttcgcccgctaccccgaccacatgaagcagcacgacttcttcaagtccgccatgcccgaaggctacgtccaggagcgcaccatcttcttcaaggacgacggcaactacaagacccgcgccgaggtgaagttcgagggcgacaccctggtgaaccgcatcgagctgaagggcatcggcttcaaggaggacggcaacatcctggggcacaagctggagtacaaccgtggtggtagccctaccgcgaaagatcgtattctggcgagccgtttaggtgcacctgcggttgaagcgttagttggtggtgcgagcggcgttatggttggtgaagtggaaggcgaagtggatctgaccccgctgaaagaagcagttgaacgccgcaaagatattaaccgcgcgttactgcgcttatcacaggtgctggcgtta

SEQ ID NO: 12 - protein, 568 aa, synthetic construct
MKRIGVFTSGGDAPGMNAAIRAVVRQAHALGVEVIGIRRGYAGMIQGEMVPLGVRDVANIIQRGGTILLTARSQEFLTEEGRAKAYAKLQAAGIEGLVAIGGDGTFRGALFLVEEHGMPVVGVPGTIDNDLYGTDYTIGFDTAVNTALEAIDRIRDTAASHERVFFIEVMGRHAGFIALDVGLAGGAEVIAVPEEPVDPKAVAEVLEASQRRGKKSSIVVVAEGAYPGGAAGLLAAIREHLQVEARVTVLGHKLSNSDNVYIMADKQKNGIKANFKIRHNVEDGSVQLADHYQQNTPIGDGPVLLPDNHYLSFQSVLSKDPNEKRDHMVLLEFVTAAGITLGMDELYNVDGGSGGTGSKGEELFTGVVPILVELDGDVNGHKFSVSGEGEGDATYGKLTLKLICTTGKLPVPWPTLVTTLGYGLKCFARYPDHMKQHDFFKSAMPEGYVQERTIFFKDDGNYKTRAEVKFEGDTLVNRIELKGIGFKEDGNILGHKLEYNLFGSPTAKDRILASRLGAPAVEALVGGASGVMVGEVEGEVDLTPLKEAVERRKDINRALLRLSQVLAL

SEQ ID NO: 13 - DNA, 1704 bp, synthetic construct
  source 1..1704: mol_type = other DNA
atgaaacgcattggcgtgtttaccagcggtggtgatgcgcctggtatgaatgcggcgattcgtgcggttgttcgtcaggcgcatgcgttaggcgttgaagtgattggcattcgccgtggctatgcgggtatgattcagggtgaaatggtgcctttaggcgtgcgtgatgtggcgaacattattcaacgcggcggcaccattttattaaccgcgcgcagccaagaatttctgaccgaagaaggccgcgcaaaagcgtatgcgaaactgcaggcggcgggtattgaaggtctggtggcgattggtggtgatggaacctttcgtggcgcgctgtttctggtggaagaacatggcatgccggttgtgggtgtgcctggaaccattgataacgatctgtacggcaccgattataccattggctttgataccgcggttaacacagccctggaagcgattgatcgcattcgtgataccgcggcgtcacatgaacgcgtgtttttcattgaagtgatgggccgccatgcgggttttattgcgctggatgttggcttagcaggcggtgcggaagttattgcggtgccggaagaacctgtggacccgaaagcggtggcggaagttttagaagcgagccaacgccgtggcaaaaaaagcagcattgtggtggttgcggaaggtgcatatcctggtggcgcggcgggtttattagcggcgattcgcgaacatctgcaggttgaagcgcgcgttaccgtgttaggccataagttgtcgaacagcgacaacgtctatatcatggccgacaagcagaagaacggcatcaaggccaacttcaagatccgccacaacgtcgaggacggcagcgtgcagctcgccgaccactaccagcagaacacccccatcggcgacggccccgtgctgctgcccgacaaccactacctgagcttccagtccgtcctgagcaaagaccccaacgagaagcgcgatcacatggtcctgctggagttcgtgaccgccgccgggatcactctcggcatggacgagctgtacaacgtggatggcggtagcggtggcaccggcagcaagggcgaggagctgttcaccggggtggtgcccatcctggtcgagctggacggcgacgtaaacggccacaagttcagcgtgtccggcgagggcgagggcgatgccacctacggcaagctgaccctgaagctgatctgcaccaccggcaagctgcccgtgccctggcccaccctcgtgaccaccctcggctacggcctgaagtgcttcgcccgctaccccgaccacatgaagcagcacgacttcttcaagtccgccatgcccgaaggctacgtccaggagcgcaccatcttcttcaaggacgacggcaactacaagacccgcgccgaggtgaagttcgagggcgacaccctggtgaaccgcatcgagctgaagggcatcggcttcaaggaggacggcaacatcctggggcacaagctggagtacaatttgtttggtagccctaccgcgaaagatcgtattctggcgagccgtttaggtgcacctgcggttgaagcgttagttggtggtgcgagcggcgttatggttggtgaagtggaaggcgaagtggatctgaccccgctgaaagaagcagttgaacgccgcaaagatattaaccgcgcgttactgcgcttatcacaggtgctggcgtta